European Patent Specification EP 3 431 586 B1, published July 10, 2024. Title: Highly functional hepatocytes and use thereof. Applicant: YONEMITSU, Yoshikazu GAIA BioMedicine Inc. The sequence listing filed with the application follows.

SEQUENCE LISTING (10 sequences)

SEQ ID NO: 1 - DNA, 26 bp, Artificial Sequence
  PCR primer, hALB For
cctttggcacaatgaagtgggtaacc

SEQ ID NO: 2 - DNA, 25 bp, Artificial Sequence
  PCR primer, hALB Rev
cagcagtcagccatttcaccatagg

SEQ ID NO: 3 - DNA, 27 bp, Artificial Sequence
  PCR primer, hHNF4a For
ctgctcggagccaccaagagatccatg

SEQ ID NO: 4 - DNA, 25 bp, Artificial Sequence
  PCR primer, hHNF4a Rev
atcatctgccacgtgatgctctgca

SEQ ID NO: 5 - DNA, 25 bp, Artificial Sequence
  PCR primer, hOCT4 For
gacaacaatgaaaatcttcaggaga

SEQ ID NO: 6 - DNA, 23 bp, Artificial Sequence
  PCR primer, hOCT4 Rev
ttctggcgccggttacagaacca

SEQ ID NO: 7 - DNA, 22 bp, Artificial Sequence
  PCR primer, hCYP3A4 For
ccttacatatacacaccctttg

SEQ ID NO: 8 - DNA, 23 bp, Artificial Sequence
  PCR primer, hCYP3A4 Rev
ggttgaagaagtcctcctaagct

SEQ ID NO: 9 - DNA, 19 bp, Artificial Sequence
  PCr primer, h À-actin For
tcaccaccacggccgagcg

SEQ ID NO: 10 - DNA, 20 bp, Artificial Sequence
  PCR primer, h À-actin Rev
tctccttctgcatcctgtcg